European Patent Application EP 4 674 949 A1, published January 7, 2026. Title: A Growth-promoting probiotic strain and use thereof. Applicant: Inner Mongolia Mengniu Dairy (Group) Co., Ltd. Application EP. The sequence listing filed with the application follows.

SEQUENCE LISTING (3 sequences)

SEQ ID NO: 1 - DNA, 20 bp, synthetic construct
  source 1..20: mol_type = other DNA
agagtttgatcmtggctcag

SEQ ID NO: 2 - DNA, 19 bp, synthetic construct
  source 1..19: mol_type = other DNA
ggttaccttgttacgactt

SEQ ID NO: 3 - DNA, 1437 bp, Lactiplantibacillus plantarum
  source 1..1437: mol_type = genomic DNA
gcagtcgaacgaactctggtattgattggtgcttgcatcatgatttacatttgagtgagtggcgaactggtgagtaacacgtgggaaacctgcccagaagcgggggataacacctggaaacagatgctaataccgcataacaacttggaccgcatggtccgagcttgaaagatggcttcggctatcacttttggatggtcccgcggcgtattagctagatggtggggtaacggctcaccatggcaatgatacgtagccgacctgagagggtaatcggccacattgggactgagacacggcccaaactcctacgggaggcagcagtagggaatcttccacaatggacgaaagtctgatggagcaacgccgcgtgagtgaagaagggtttcggctcgtaaaactctgttgttaaagaagaacatatctgagagtaactgttcaggtattgacggtatttaaccagaaagccacggctaactacgtgccagcagccgcggtaatacgtaggtggcaagcgttgtccggatttattgggcgtaaagcgagcgcaggcggttttttaagtctgatgtgaaagccttcggctcaaccgaagaagtgcatcggaaactgggaaacttgagtgcagaagaggacagtggaactccatgtgtagcggtgaaatgcgtagatatatggaagaacaccagtggcgaaggcggctgtctggtctgtaactgacgctgaggctcgaaagtatgggtagcaaacaggattagataccctggtagtccataccgtaaacgatgaatgctaagtgttggagggtttccgcccttcagtgctgcagctaacgcattaagcattccgcctggggagtacggccgcaaggctgaaactcaaaggaattgacgggggcccgcacaagcggtggagcatgtggtttaattcgaagctacgcgaagaaccttaccaggtcttgacatactatgcaaatctaagagattagacgttcccttcggggacatggatacaggtggtgcatggttgtcgtcagctcgtgtcgtgagatgttgggttaagtcccgcaacgagcgcaacccttattatcagttgccagcattaagttgggcactctggtgagactgccggtgacaaaccggaggaaggtggggatgacgtcaaatcatcatgccccttatgacctgggctacacacgtgctacaatggatggtacaacgagttgcgaactcgcgagagtaagctaatctcttaaagccattctcagttcggattgtaggctgcaactcgcctacatgaagtcggaatcgctagtaatcgcggatcagcatgccgcggtgaatacgttcccgggccttgtacacaccgcccgtcacaccatgagagtttgtaacacccaaagtcggtggggtaaccttttaggaaccagccgcctaa